European Patent Specification EP 3 494 227 B1, published December 11, 2024. Title: HELPER OLIGONUCLEOTIDE FOR IMPROVING EFFICIENCY OF AMPLIFICATION AND DETECTION/QUANTITATION OF NUCLEIC ACIDS. Applicant: Roche Diagnostics GmbH F. Hoffmann-La Roche AG Roche Molecular Systems, Inc. The sequence listing filed with the application follows.

SEQUENCE LISTING (5 sequences)

SEQ ID NO: 1 - DNA, 18 bp, Artificial Sequence
  Forward Primer
  modified_base (18)..(18): t-Butyl Benzyl-dC
tgggcagggtggttgctc

SEQ ID NO: 2 - DNA, 25 bp, Artificial Sequence
  Reverse Primer
  modified_base (25)..(25): t-Butyl Benzyl-dA
gttgcatagtttaccccgtcctcaa

SEQ ID NO: 3 - DNA, 25 bp, Artificial Sequence
  Reverse Primer
  modified_base (25)..(25): t-Butyl Benzyl-dA
gttgcatagtttatcccgtcctcaa

SEQ ID NO: 4 - DNA, 25 bp, Artificial Sequence
  Probe
atcccgctcgtaggcggccccgttg

SEQ ID NO: 5 - DNA, 53 bp, Artificial Sequence
  Non-Extending Helper Oligonucleotide
gttgcatagtttatcccgtcttcaagaaccttcacaccgtgtgcgaaaaaaaa